European Patent Specification EP 3 570 878 B1, published August 12, 2026. Title: Anti-HERV-K envelope antibody and uses thereof. Applicant: GENEURO SA. The sequence listing filed with the application follows.

SEQUENCE LISTING (9 sequences)

SEQ ID NO: 1 - protein, 11 aa, Mus musculus
QSLLDSDGKTY

SEQ ID NO: 2 - protein, 3 aa, Mus musculus
LVS

SEQ ID NO: 3 - protein, 9 aa, Mus musculus
LQATHFPWT

SEQ ID NO: 4 - protein, 8 aa, Mus musculus
GYTFTSYW

SEQ ID NO: 5 - protein, 8 aa, Mus musculus
IDPYDSET

SEQ ID NO: 6 - protein, 10 aa, Mus musculus
ASLYYYGISL

SEQ ID NO: 7 - protein, 112 aa, Mus musculus
DVVMTQTPLTLSVTIGQPASISCKSSQSLLDSDGKTYLNWLLQRPGESPKLLIYLVSKLDSGVPDRFTGSGSGTDFTLKISRVEAEDLGVYYCLQATHFPWTFGGGTKLEIK

SEQ ID NO: 8 - protein, 116 aa, Mus musculus
QVQLQQPGAELVRPGASVKLSCKASGYTFTSYWMNWVKQRPEQGLEWIGRIDPYDSETHYNQKFKDKAILTVDKSSSTAYMQLSSLTSEDSAVYYCASLYYYGISLWGQGTLVTVS

SEQ ID NO: 9 - protein, 15 aa, Homo sapiens
SLDKHKHKKLQSFYP